European Patent Specification EP 4 114 977 B1, published September 11, 2024. Title: Non-invasive Successfulness Test of in vitro Fertilization Process. Applicant: Pavol Jozef Safarik University in Kosice. The sequence listing filed with the application follows.

SEQUENCE LISTING (36 sequences)

SEQ ID NO: 1 - RNA, 22 nt, Homo sapiens
  iso-hsa-miR-126-3p
cgtaccgtgagaaataatgcgt

SEQ ID NO: 2 - RNA, 22 nt, Homo sapiens
  iso-hsa-let-7i-5p
tgtggtagtagtttgtgctgta

SEQ ID NO: 3 - RNA, 25 nt, Homo sapiens
  iso-hsa-miR-342-3p
tctcacacagaaatcggacccgtct

SEQ ID NO: 4 - RNA, 22 nt, Homo sapiens
  iso-hsa-let-7b-5p
tgaggtagtaggttgtgtgtta

SEQ ID NO: 5 - RNA, 23 nt, Homo sapiens
  iso-hsa-miR-132-3p
taacagcctacagccatggtcgt

SEQ ID NO: 6 - RNA, 23 nt, Homo sapiens
  iso-hsa-miR-23b-3p
gcacattgccagggattaccact

SEQ ID NO: 7 - RNA, 22 nt, Homo sapiens
  iso-hsa-miR-125a-5p
tccctgagaccttttaacctgt

SEQ ID NO: 8 - RNA, 19 nt, Homo sapiens
  iso-hsa-miR-584-5p
tatggtttgcctgggactg

SEQ ID NO: 9 - RNA, 25 nt, Homo sapiens
  iso-hsa-miR-127-3p
tcggatcagtctgagcttggctttt

SEQ ID NO: 10 - RNA, 20 nt, Homo sapiens
  iso-hsa-miR-101-3p
tacactactgtgataactga

SEQ ID NO: 11 - RNA, 24 nt, Homo sapiens
  iso-hsa-miR-151a-3p
tactagactaaagctccttgaggt

SEQ ID NO: 12 - RNA, 23 nt, Homo sapiens
  iso-hsa-miR-92a-3p
gattgcacttgtcccggcctgaa

SEQ ID NO: 13 - RNA, 20 nt, Homo sapiens
  iso-hsa-let-7b-5p
tgaggtagtatgttgtgtgg

SEQ ID NO: 14 - RNA, 23 nt, Homo sapiens
  iso-hsa-miR-589-5p
tgagaaccacgtccgctctgagc

SEQ ID NO: 15 - RNA, 22 nt, Homo sapiens
  iso-hsa-miR-652-3p
gatggcgccactagggttgtga

SEQ ID NO: 16 - RNA, 23 nt, Homo sapiens
  iso-hsa-miR-1307-3p
actcggcgtagcgtcggtcgtgt

SEQ ID NO: 17 - RNA, 21 nt, Homo sapiens
  iso-hsa-miR-382-5p
gaagttgttcgcggtggattc

SEQ ID NO: 18 - RNA, 23 nt, Homo sapiens
  iso-hsa-let-7b-5p
tgaggtagtaagttgtgtggtat

SEQ ID NO: 19 - RNA, 24 nt, Homo sapiens
  iso-hsa-let-7i-5p
tgagttagtagtttgtgctgtttt

SEQ ID NO: 20 - RNA, 21 nt, Homo sapiens
  iso-hsa-let-7b-5p
tgaggtggtaggttgtgtggt

SEQ ID NO: 21 - RNA, 23 nt, Homo sapiens
  iso-hsa-miR-423-5p
tgaggggcagagagcgagactta

SEQ ID NO: 22 - RNA, 23 nt, Homo sapiens
  iso-hsa-miR-21-5p
tagcttaccagactgatgttgac

SEQ ID NO: 23 - RNA, 23 nt, Homo sapiens
  iso-hsa-miR-486-5p
tcctgtactgagctgcccagaga

SEQ ID NO: 24 - RNA, 22 nt, Homo sapiens
  iso-hsa-miR-486-5p
tcctgtactgagctgcctcgag

SEQ ID NO: 25 - RNA, 22 nt, Homo sapiens
  iso-hsa-miR-25-3p
cattgcaattgtctcggtctga

SEQ ID NO: 26 - RNA, 21 nt, Homo sapiens
  iso-hsa-miR-3613-5p
tgttgtacttttttttttgtt

SEQ ID NO: 27 - RNA, 23 nt, Homo sapiens
  iso-hsa-miR-142-3p
tgtagtgtttcctaccttatgga

SEQ ID NO: 28 - RNA, 23 nt, Homo sapiens
  iso-hsa-miR-664a-5p
actggctagggaaaatgattgga

SEQ ID NO: 29 - RNA, 21 nt, Homo sapiens
  iso-hsa-miR-151a-3p
caagactgaagctccttgagg

SEQ ID NO: 30 - RNA, 22 nt, Homo sapiens
  iso-hsa-miR-92a-3p
tatcgcacttgtcccggcctgt

SEQ ID NO: 31 - RNA, 20 nt, Homo sapiens
  iso-hsa-let-7a-5p
tgatgtagtaggttgtatag

SEQ ID NO: 32 - RNA, 24 nt, Homo sapiens
  iso-hsa-let-7b-5p
tgaggtagtaggttgtgtggttta

SEQ ID NO: 33 - RNA, 21 nt, Homo sapiens
  iso-hsa-miR-100-5p
aacccgtagatccgaacttgt

SEQ ID NO: 34 - RNA, 23 nt, Homo sapiens
  iso-hsa-miR-191-5p
caatggaatcccaaaagcagctg

SEQ ID NO: 35 - RNA, 20 nt, Homo sapiens
  iso-hsa-let-7a-5p
tgagttagtaggttgtatag

SEQ ID NO: 36 - RNA, 22 nt, Homo sapiens
  iso-hsa-let-7d 5p
agaggtagtaggttgcgtagtt